European Patent Application EP 4 209 508 A1, published July 12, 2023. Title: Development of Nanobodies as first-in-class inhibitors for the deNEDDylating enzyme NEDP1. Applicant: CNRS PARIS UNIV MONTPELLIER UNIV VRIJE. The sequence listing filed with the application follows.

SEQUENCE LISTING (109 sequences)

SEQ ID NO: 1 - protein, 8 aa, artificial
  CDR1 R2DP44
GSILRINV

SEQ ID NO: 2 - protein, 7 aa, Artificial Sequence
  CDR2 R2DP44
ITSGGST

SEQ ID NO: 3 - protein, 6 aa, Artificial Sequence
  CDR3 R2DP44
AAAGGS

SEQ ID NO: 4 - protein, 8 aa, Artificial Sequence
  CDR1 R2DP58
GSIRSINV

SEQ ID NO: 5 - protein, 7 aa, Artificial Sequence
  CDR2 R2DP58
ITSGGYT

SEQ ID NO: 6 - protein, 6 aa, Artificial Sequence
  CDR3 R2DP58
KGVAVP

SEQ ID NO: 7 - protein, 8 aa, Artificial Sequence
  CDR1 R2DP61
KSIFSINV

SEQ ID NO: 8 - protein, 7 aa, Artificial Sequence
  CDR2 R2DP61
VTSGGST

SEQ ID NO: 9 - protein, 9 aa, Artificial Sequence
  CDR3 R2DP61
AAVERGMDY

SEQ ID NO: 10 - protein, 8 aa, Artificial Sequence
  CDR1 R2DP80
GSIFKINV

SEQ ID NO: 11 - protein, 7 aa, Artificial Sequence
  CDR2 R2DP80
ITSGGST

SEQ ID NO: 12 - protein, 6 aa, Artificial Sequence
  CDR3 R2DP80
ATPGSV

SEQ ID NO: 13 - protein, 8 aa, Artificial Sequence
  CDR1 R2DP16
GSDFSINV

SEQ ID NO: 14 - protein, 7 aa, Artificial Sequence
  CDR2 R2DP16
ISGGGAT

SEQ ID NO: 15 - protein, 9 aa, Artificial Sequence
  CDR3 R2DP16
RGIVAGADY

SEQ ID NO: 16 - protein, 8 aa, Artificial Sequence
  CDR1 R2DP23
GSIASINV

SEQ ID NO: 17 - protein, 7 aa, Artificial Sequence
  CDR2 R2DP23
VANGGQS

SEQ ID NO: 18 - protein, 10 aa, Artificial Sequence
  CDR3 R2DP23
IDLEGLRIGN

SEQ ID NO: 19 - protein, 8 aa, Artificial Sequence
  CDR1 R2DP47
GSISSINV

SEQ ID NO: 20 - protein, 7 aa, Artificial Sequence
  CDR2 R2DP47
ISSFGIT

SEQ ID NO: 21 - protein, 6 aa, Artificial Sequence
  CDR3 R2DP47
KGPNTD

SEQ ID NO: 22 - protein, 8 aa, Artificial Sequence
  CDR1 R2DP49
GIIDSINV

SEQ ID NO: 23 - protein, 7 aa, Artificial Sequence
  CDR2 R2DP49
ITSRGIT

SEQ ID NO: 24 - protein, 7 aa, Artificial Sequence
  CDR3 R2DP49
TYLGRTS

SEQ ID NO: 25 - protein, 8 aa, Artificial Sequence
  CDR1 R2DP69
GSIFHINL

SEQ ID NO: 26 - protein, 7 aa, Artificial Sequence
  CDR2 R2DP69
ITGGGST

SEQ ID NO: 27 - protein, 10 aa, Artificial Sequence
  CDR3 R2DP69
RGLVPGKDDY

SEQ ID NO: 28 - protein, 8 aa, Artificial Sequence
  CDR1 R2DP19
GSIFSQNV

SEQ ID NO: 29 - protein, 7 aa, Artificial Sequence
  CDR2 R2DP19
ITSGGNT

SEQ ID NO: 30 - protein, 9 aa, Artificial Sequence
  CDR3 R2DP19
AGSSWVNDY

SEQ ID NO: 31 - protein, 8 aa, Artificial Sequence
  CDR1 R2DP93
GSIFSINV

SEQ ID NO: 32 - protein, 7 aa, Artificial Sequence
  CDR2 R2DP93
IINAGTT

SEQ ID NO: 33 - protein, 9 aa, Artificial Sequence
  CDR3 R2DP93
AAYLSGRTV

SEQ ID NO: 34 - protein, 8 aa, Artificial Sequence
  CDR1 R2DP11
GNIFNINV

SEQ ID NO: 35 - protein, 7 aa, Artificial Sequence
  CDR2 R2DP11
ITSGRLT

SEQ ID NO: 36 - protein, 9 aa, Artificial Sequence
  CDR3 R2DP11
AAARPGGYY

SEQ ID NO: 37 - protein, 8 aa, Artificial Sequence
  CDR1 R2DP46
GSPFSIGT

SEQ ID NO: 38 - protein, 7 aa, Artificial Sequence
  CDR2 R2DP46
ITRGGAT

SEQ ID NO: 39 - protein, 9 aa, Artificial Sequence
  CDR3 R2DP46
SVWAGDRAY

SEQ ID NO: 40 - protein, 8 aa, Artificial Sequence
  CDR1 R2DP67
GSPFSIGT

SEQ ID NO: 41 - protein, 7 aa, Artificial Sequence
  CDR2 R2DP67
ITRGGAT

SEQ ID NO: 42 - protein, 9 aa, Artificial Sequence
  CDR3 R2DP67
SVWAGDRAF

SEQ ID NO: 43 - protein, 8 aa, Artificial Sequence
  CDR1 R2DP34
GSATRINV

SEQ ID NO: 44 - protein, 7 aa, Artificial Sequence
  CDR2 R2DP34
VTSGGST

SEQ ID NO: 45 - protein, 9 aa, Artificial Sequence
  CDR3 R2DP34
AAVEDEYVY

SEQ ID NO: 46 - protein, 8 aa, Artificial Sequence
  CDR1 R2DP78
GITFTLNV

SEQ ID NO: 47 - protein, 7 aa, Artificial Sequence
  CDR2 R2DP78
ISNGAIS

SEQ ID NO: 48 - protein, 9 aa, Artificial Sequence
  CDR3 R2DP78
ATVIGGSRF

SEQ ID NO: 49 - protein, 8 aa, Artificial Sequence
  CDR1 R2DP12
GSTSSFNV

SEQ ID NO: 50 - protein, 7 aa, Artificial Sequence
  CDR2 R2DP12
ITSGGIT

SEQ ID NO: 51 - protein, 9 aa, Artificial Sequence
  CDR3 R2DP12
GGVVDGRVY

SEQ ID NO: 52 - protein, 8 aa, Artificial Sequence
  CDR1 R2DP57
GTTSSFNV

SEQ ID NO: 53 - protein, 7 aa, Artificial Sequence
  CDR2 R2DP57
ITSGGST

SEQ ID NO: 54 - protein, 9 aa, Artificial Sequence
  CDR3 R2DP57
GGVVGGRVY

SEQ ID NO: 55 - protein, 8 aa, Artificial Sequence
  CDR1 R2DP62
GSIVSSNA

SEQ ID NO: 56 - protein, 7 aa, Artificial Sequence
  CDR2 R2DP62
IANSGIT

SEQ ID NO: 57 - protein, 9 aa, Artificial Sequence
  CDR3 R2DP62
AAIFNQQFA

SEQ ID NO: 58 - protein, 8 aa, Artificial Sequence
  CDR1 R2DP35
GVMFSTGV

SEQ ID NO: 59 - protein, 7 aa, Artificial Sequence
  CDR2 R2DP35
ITSGGLT

SEQ ID NO: 60 - protein, 5 aa, Artificial Sequence
  CDR3 R2DP35
NVRGY

SEQ ID NO: 61 - protein, 8 aa, Artificial Sequence
  CDR1 R2DP55
GFTFDDHA

SEQ ID NO: 62 - protein, 8 aa, Artificial Sequence
  CDR2 R2DP55
LSNSDGTT

SEQ ID NO: 63 - protein, 17 aa, Artificial Sequence
  CDR3 R2DP55
AICHFRERDGSAWFEGS

SEQ ID NO: 64 - protein, 112 aa, Artificial Sequence
  R2DP44 aa sequence
QVQLQESGGGLVQPGGSLRLSCAASGSILRINVMGWYRQASGKQRESVAAITSGGSTTYANSVRGRFTISRDNAKNTVYLQMNSLKPEDTAVYYCAAAGGSWGQGTQVTVSS

SEQ ID NO: 65 - protein, 112 aa, Artificial Sequence
  R2DP58 aa sequence
QVQLQESGGGLVQPGGSLRLSCAASGSIRSINVMGWYRQAPGKQRELVAGITSGGYTNYADSVKGRFTISRDNAKNTVYLQMNSLKPEDTAVYYCKGVAVPWGQGTQVTVSS

SEQ ID NO: 66 - protein, 115 aa, Artificial Sequence
  R2DP61 aa sequence
QVQLQESGGGLVQAGGSLRLSCAASKSIFSINVMGWYRQAPGKQRESVAAVTSGGSTNYRDSVKGRFTISRDNAKNTVYLQMNRLKPEDTAVYYCAAVERGMDYWGQGTQVTVSS

SEQ ID NO: 67 - protein, 112 aa, Artificial Sequence
  R2DP80 aa sequence
QVQLQESGGGLVQAGGSLRLSCAASGSIFKINVMAWYRQAPGKQRESVAAITSGGSTNYAASVKGRFVISRDNAKNTVYLQMDSLKPEDTAVYYCATPGSVPGQGTQVTVSS

SEQ ID NO: 68 - protein, 115 aa, Artificial Sequence
  R2DP16 aa sequence
QVQLQESGGGLVQPGGSLRLSCAASGSDFSINVMGWYRQAPGKERESVATISGGGATAYAYSVKGRFTISRDNAKNTVYLQMNKLKPEDTAVYFCRGIVAGADYWGQGTQVTVSS

SEQ ID NO: 69 - protein, 116 aa, Artificial Sequence
  R2DP23 aa sequence
QVQLQESGGGLVQPGGSLRLSCAASGSIASINVMAWYRQAPGKQRESVAAVANGGQSTYADSVKGRFTISRDNAKNTMYLQMNSLKPEDTAVYYCIDLEGLRIGNWGQGTQVTVSS

SEQ ID NO: 70 - protein, 112 aa, Artificial Sequence
  R2DP47 aa sequence
QVQLQESGGGLVEPGGSLRLSCAASGSISSINVMAWYRQAPGKQRESVAAISSFGITTYSETVKGRFTASRDNAKNTMYLQMNNLKPEDTAVYYCKGPNTDWGQGTQVTVSS

SEQ ID NO: 71 - protein, 113 aa, Artificial Sequence
  R2DP49 aa sequence
QVQLQESGGGLVQPGGSLRLSCAASGIIDSINVMAWYRQAPGKQRESVATITSRGITAYADSVKGRFIISRDNAKNTMYLQMNSLKPEDTAVYYCTYLGRTSWGQGTQVTVSS

SEQ ID NO: 72 - protein, 116 aa, Artificial Sequence
  R2DP69 aa sequence
QVQLQESGGGLVQPRGSLRLSCAASGSIFHINLMGWYRQAPGKQRESVAVITGGGSTTYRDSVKGRFTISRDNAKNTVYLQMNSLKPEDTGVYYCRGLVPGKDDYWGQGTQVTVSS

SEQ ID NO: 73 - protein, 115 aa, Artificial Sequence
  R2DP19 aa sequence
QVQLQESGGGLVQAGGSLRLSCVVSGSIFSQNVMGWYRQAPGKQRESVAAITSGGNTNYRDSVKGRFTISRDNAKDTVYLQMNRLKPEDTAVYYCAGSSWVNDYWGQGTQVTVSS

SEQ ID NO: 74 - protein, 115 aa, Artificial Sequence
  R2DP93 aa sequence
QVQLQESGGGLVQAGGSLRLSCAASGSIFSINVMAWYRQAPGKQREAVASIINAGTTIYANSVKGRFTISRDNVKNALYLQMNSLKPEDTAVYYCAAYLSGRTVWGQGTQVTVSS

SEQ ID NO: 75 - protein, 115 aa, Artificial Sequence
  R2DP11 aa sequence
QVQLQESGGGLVQAGGSLRLSCVASGNIFNINVMAWYRQPPGKQRESVAAITSGRLTTYNASVKGRFTIYRDNAENTVYLQMNGLKPEDTGVYYCAAARPGGYYWGQGTQVTVSS

SEQ ID NO: 76 - protein, 115 aa, Artificial Sequence
  R2DP46 aa sequence
QVQLQESGGGLVQAGGSLRLSCAASGSPFSIGTMAWYRQAPGNQRASVAAITRGGATTYANSVKGRFTVSRDNAKNTVYLQMNSLKPEDTAAYYCSVWAGDRAYWGQGTQVTVSS

SEQ ID NO: 77 - protein, 115 aa, Artificial Sequence
  R2DP67 aa sequence
QVQLQESGGGLVQAGGSLRLSCAASGSPFSIGTMAWYRQAPGNQRASVAAITRGGATTYANSVKGRFTVSRDNAKNTVYLQMNSLKPEDTAVYYCSVWAGDRAFWGQGTQVTVSS

SEQ ID NO: 78 - protein, 115 aa, Artificial Sequence
  R2DP34 aa sequence
QVQLQESGGGLVQAGGSLRLSCAASGSATRINVMSWYRQAPGKKRESVAVVTSGGSTNYLASVKGRFTISRDNAKNTVYLQMNSLKPEDTAVYYCAAVEDEYVYWGKGTQVTVSS

SEQ ID NO: 79 - protein, 115 aa, Artificial Sequence
  R2DP78 aa sequence
QVQLQESGGGLVQAGGSLRLSCAASGITFTLNVMGWYRQAPGKQREAVATISNGAISNYANSVKGRFTISRDNAKNTVYLQMNSLKPEDTAVYYCATVIGGSRFAGQGTQVTVSS

SEQ ID NO: 80 - protein, 115 aa, Artificial Sequence
  R2DP12 aa sequence
QVQLQESGGGLVQAGGSLRLSCAASGSTSSFNVMAWYHQAPGKQRESVASITSGGITVYRDSVKGRFAISSDNAKNTVFLQMNSLKPEDTGVYYCGGVVDGRVYRGQGTQVTVSS

SEQ ID NO: 81 - protein, 115 aa, Artificial Sequence
  R2DP57 aa sequence
QVQLQESGGGLVQAGGSLRLSCAVSGTTSSFNVMNWHHQAPGKQRESVASITSGGSTLYRDSVKGRLTISRDNAKNAVYLQMNSLKPEDTGVYYCGGVVGGRVYWGQGTQVTVSS

SEQ ID NO: 82 - protein, 115 aa, Artificial Sequence
  R2DP62 aa sequence
QVQLQESGGGLVQAGGSLRLSCAASGSIVSSNAMSWYRQAPGKQRESVAAIANSGITTYRDSVKGRFTISRDNTKNTMYLQMNSLRPEDTAVYYCAAIFNQQFAWGQGTQVTVSS

SEQ ID NO: 83 - protein, 111 aa, Artificial Sequence
  R2DP35 aa sequence
QVQLQESGGGLVQPGGSLTLSCAASGVMFSTGVMGWYRQAPGKQREAVAAITSGGLTTYKDSVKGRFAISRDNTKSTGYLQMNRLRPEDTAVYYCNVRGYWGQGTQVTVSS

SEQ ID NO: 84 - protein, 124 aa, Artificial Sequence
  R2DP55 aa sequence
QVQLQESGGGLVQAGGSLRVSCATSGFTFDDHAIGWFRQAPGKEREAVSCLSNSDGTTYYTDSVKGRFTASSDNAKKTGYLQMKSLKPEDTAVYYCAICHFRERDGSAWFEGSWGQGTQVTVSS

SEQ ID NO: 85 - DNA, 384 bp, Artificial Sequence
  R2DP44 nucleic acid sequence
caggtgcagctgcaggagtctgggggaggcttggtgcagcctggggggtctctgagactctcctgtgcagcctctggaagcatcttacgtatcaatgtcatgggctggtaccgccaggcttcagggaagcagcgggagtcggtcgcagctattactagtggtggtagcacaacgtatgcaaactccgtgaggggccgattcaccatctccagagacaacgccaagaacacggtgtatctgcaaatgaacagcctgaaacctgaggacacagccgtctattactgtgcagccgccgggggttcctggggccaggggacccaggtcaccgtctccagcggccgctacccgtacgacgttccggactacggttccggccgagcatag

SEQ ID NO: 86 - DNA, 384 bp, Artificial Sequence
  R2DP58 nucleic acid sequence
caggtgcagctgcaggagtctgggggaggcttggtgcagcctggggggtctctgagactctcctgtgcagcctctggaagcatccgcagtatcaatgtaatgggctggtaccgccaggctccagggaagcagcgcgagttggtcgcaggtattactagtggtggttacacaaactatgcagactccgtgaagggccgattcaccatctccagagacaacgccaagaacacggtgtatctgcaaatgaacagcctgaaacctgaggacacggccgtctattactgcaagggggtagctgttccctggggccaggggacccaggtcaccgtctccagcggccgctacccgtacgacgttccggactacggttccggccgagcatag

SEQ ID NO: 87 - DNA, 393 bp, Artificial Sequence
  R2DP61 nucleic acid sequence
caggtgcagctgcaggagtctgggggaggcttggtgcaggctggggggtctctgagactctcctgtgcagcctctaaaagcatcttcagtatcaatgtcatgggctggtaccgccaggctccagggaagcagcgcgagtctgtcgcagctgttactagtggtggaagcacaaactatcgagactccgtgaagggccgattcaccatctccagagataacgccaagaacacggtgtatctgcaaatgaaccgcctgaaacctgaggacacagccgtctattactgtgcagcagttgaaagggggatggactactggggccaggggacccaggtcaccgtctccagcggccgctacccgtacgacgttccggactacggttccggccgagcatag

SEQ ID NO: 88 - DNA, 384 bp, Artificial Sequence
  R2DP80 nucleic acid sequence
caggtgcagctgcaggagtctgggggaggcttggtgcaggctggggggtctctgagactctcctgtgcagcctctggaagcatcttcaagatcaatgtcatggcctggtaccgccaggctccagggaagcagcgcgagtcggtcgcagctattactagtggtggtagcacaaactatgcagcatccgtgaagggccgattcgtcatctccagagacaacgccaagaacacggtgtatctgcaaatggacagcctgaaacctgaggacacagccgtctattactgtgcaaccccggggtccgtccccggacaggggacccaggtcaccgtctccagcggccgctacccgtacgacgttccggactacggttccggccgagcatag

SEQ ID NO: 89 - DNA, 393 bp, Artificial Sequence
  R2DP16 nucleic acid sequence
caggtgcagctgcaggagtctgggggaggcttggtgcagcctggggggtctctgagactctcctgtgcggcctctggaagcgacttcagtatcaatgtcatgggctggtaccgccaggctccagggaaggagcgcgaatcggtcgcaaccatttccggtggaggtgcgactgcctatgcatactccgtgaagggccgattcaccatttccagagacaacgccaagaacacggtgtatctgcaaatgaacaaactgaaaccagaggacacggccgtctatttttgtcgagggatagtagctggtgcagactactggggccaggggacccaggtcaccgtctccagcggccgctacccgtacgacgttccggactacggttccggccgagcatag

SEQ ID NO: 90 - DNA, 396 bp, Artificial Sequence
  R2DP23 nucleic acid sequence
caggtgcagctgcaggagtctgggggaggcttggtgcagcctggagggtctctgagactctcctgcgcagcctctggaagcatcgctagtatcaatgtcatggcctggtaccgccaggctccagggaagcagcgcgagtcggtcgcagctgttgctaatggtggtcaatcaacctatgcagactccgtgaagggccgattcaccatctccagagacaacgccaagaacacgatgtatctgcaaatgaacagcctgaaacctgaggacacggccgtctattactgtatagatttagaaggactacgcattgggaactggggccaggggacccaggtcaccgtctccagcggccgctacccgtacgacgttccggactacggttccggccgagcatag

SEQ ID NO: 91 - DNA, 384 bp, Artificial Sequence
  R2DP47 nuceic acid sequence
caggtgcagctgcaggagtctgggggaggcttggtggagcctggggggtctctgagactctcctgtgcagcctctggaagcatctccagtatcaatgtcatggcctggtaccgccaggctccagggaagcagcgcgagtcggtcgcagcaattagtagttttggtatcacaacctactcagagaccgtgaagggccgattcaccgcctccagagacaatgccaagaacacgatgtatctgcaaatgaacaacctgaaacctgaggacacggccgtctattactgtaaaggaccaaatacagactggggccaggggacccaggtcaccgtctccagcggccgctacccgtacgacgttccggactacggttccggccgagcatag

SEQ ID NO: 92 - DNA, 387 bp, Artificial Sequence
  R2DP49  nucleic acid sequence
caggtgcagctgcaggagtctgggggaggcttggtgcagcctggggggtctctgagactctcctgtgcagcctctggaatcatcgacagtatcaatgtcatggcctggtaccgccaggctccagggaagcagcgcgagtcggtcgcgactattactagtagaggtattactgcctatgcagactccgtgaagggccgattcatcatctccagagacaacgccaagaacacgatgtatctgcaaatgaacagcctgaaacctgaggacacggccgtctattactgcacatatttaggccggaccagctggggccaggggacccaggtcaccgtctccagcggccgctacccgtacgacgttccggactacggttccggccgagcatag

SEQ ID NO: 93 - DNA, 396 bp, Artificial Sequence
  R2DP69 nucleic acid sequence
caggtgcagctgcaggagtctggaggaggcttggtgcagcctagggggtctctgagactctcctgtgcagcctctggaagcatcttccatatcaatctcatgggctggtaccgccaggctccagggaagcagcgcgagtcggtcgcagttattactggtggtggttctacaacctatcgagactccgtgaagggccgattcaccatctccagagacaacgccaagaacacggtgtatctgcaaatgaacagcctgaaacctgaagacacaggtgtctattactgtagaggattagtacctggtaaggatgactactggggccaggggacccaggtcaccgtctccagcggccgctacccgtacgacgttccggactacggttccggccgagcatag

SEQ ID NO: 94 - DNA, 393 bp, Artificial Sequence
  R2DP19 nucleic acid sequence
caggtgcagctgcaggagtctgggggaggcttggtgcaggctggggggtctctgagactctcctgtgtagtatctggaagcatcttcagtcagaatgttatgggctggtaccgccaggctccagggaaacagcgcgagtcggtcgcagctattactagtggcggtaacacaaattatagagactccgtgaagggccgattcaccatctccagagacaacgccaaggatacggtgtatctgcaaatgaacagactgaaacctgaggacacagccgtctattactgtgcaggaagttcctgggttaatgactactggggccaggggacccaggtcaccgtctccagcggccgctacccgtacgacgttccggactacggttccggccgagcatag

SEQ ID NO: 95 - DNA, 393 bp, Artificial Sequence
  R2DP93 nucleic acid sequence
caggtgcagctgcaggagtctgggggaggcttggtgcaggctggggggtctctgagactctcctgtgcagcctctggaagcatcttcagtatcaatgtcatggcgtggtaccgccaggctccagggaagcagcgcgaggcggtcgcatctattattaacgccggtaccacaatctatgcaaactccgtgaagggccgattcaccatctccagagacaacgtcaagaacgctttgtatctgcaaatgaacagcctgaaaccggaggacacagccgtctattactgtgcagcatatttaagtggacgcaccgtctggggccaggggacccaggtcaccgtctccagcggccgctacccgtacgacgttccggactacggttccggccgagcatag

SEQ ID NO: 96 - DNA, 393 bp, Artificial Sequence
  R2DP11 nucleic acid sequence
caggtgcagctgcaggagtctgggggaggcttggtgcaggctggggggtctctgagactctcctgtgtagcctctggaaacatcttcaatatcaatgtcatggcctggtaccgccagcctccagggaagcagcgcgagtcggtcgcagctattactagtggtcgtctcacaacttataacgcctccgtaaagggccgattcaccatctacagagacaacgccgagaacacggtgtatctgcaaatgaacggcctgaaacctgaggacacaggtgtctattactgcgcagcagcccggccggggggatactactggggtcaggggacccaggtcaccgtctccagcggccgctacccgtacgacgttccggactacggttccggccgagcatag

SEQ ID NO: 97 - DNA, 393 bp, Artificial Sequence
  R2DP46 nucleic acid sequence
caggtgcagctgcaggagtctggaggaggcttggtgcaggctggagggtctctgagactctcctgtgcagcctctggaagtcccttcagtatcggtaccatggcctggtaccgccaggctccagggaatcagcgcgcatcggtcgcagctattactaggggtggtgcgacaacctatgcaaactccgtgaagggccgattcaccgtctctagagacaacgccaagaacacagtgtatctgcaaatgaacagcctgaaacctgaggacacggccgcctattattgtagtgtctgggccggcgatagggcctattggggccaggggacccaggtcaccgtctccagcggccgctacccgtacgacgttccggactacggttccggccgagcatag

SEQ ID NO: 98 - DNA, 393 bp, Artificial Sequence
  R2DP67 nucleic acid sequence
caggtgcagctgcaggagtctgggggaggcttggtgcaggctggagggtctctgagactctcctgtgcagcctctggaagtcccttcagtatcggtaccatggcctggtaccgccaggctccagggaatcagcgcgcatcggtcgcagctattactaggggtggtgcgacaacctatgcaaactccgtgaagggccgattcaccgtctctagagacaacgccaagaacacagtgtatctgcaaatgaacagcctgaaacctgaggacacggccgtctattattgtagtgtctgggccggcgatagggccttctggggccaggggacccaggtcaccgtctccagcggccgctacccgtacgacgttccggactacggttccggccgagcatag

SEQ ID NO: 99 - DNA, 393 bp, Artificial Sequence
  R2DP34 nucleic acid sequence
caggtgcagctgcaggagtctggaggaggcttggtgcaggctggggggtctctgagactctcctgtgcagcctctggaagcgccacgcgtatcaatgtcatgagctggtaccgccaggctcccgggaaaaagcgcgagtcggtcgcagttgtaacgagtggtggtagcacaaactatttagcgtccgtgaagggccgattcaccatctccagagacaacgccaagaacacagtgtatctgcaaatgaacagcctgaaacctgaggacacggccgtctattactgtgccgcggtcgaggatgagtatgtctactggggcaaggggacccaggtcaccgtctccagcggccgctacccgtacgacgttccggactacggttccggccgagcatag

SEQ ID NO: 100 - DNA, 393 bp, Artificial Sequence
  R2DP78 nucleic acid sequence
caggtgcagctgcaggagtctgggggaggcttggtacaggctggggggtctctgagactctcctgtgcagcctctggaatcaccttcacgctcaatgtcatgggctggtaccgccaggctccagggaagcagcgcgaggcggtcgcaactattagtaatggtgcgattagcaactatgcaaactccgtgaagggccgattcaccatctccagagacaacgccaagaacacagtgtatctgcaaatgaacagcctgaaacctgaagacacggccgtctattattgtgctacagtgatcggaggttccagatttgcaggccaggggacccaggtcaccgtctccagcggccgctacccgtacgacgttccggactacggttccggccgagcatag

SEQ ID NO: 101 - DNA, 393 bp, Artificial Sequence
  R2DP12 nucleic acid sequence
caggtgcagctgcaggagtctggaggaggcttggtgcaggctggggggtctctgagactctcctgcgcagcctctggaagcaccagcagcttcaatgtcatggcctggtaccaccaggctccagggaagcagcgcgagtcggtcgcaagtattactagtggtggtatcacagtttatagagactccgtgaagggccgcttcgccatctcaagtgacaacgccaagaacacggtgtttctgcaaatgaacagcctgaaacctgaggacacaggcgtctattactgtgggggggtagtagatgggcgagtctaccggggccaggggacccaggtcaccgtctccagcggccgctacccgtacgacgttccggactacggttccggccgagcatag

SEQ ID NO: 102 - DNA, 393 bp, Artificial Sequence
  R2DP57 nucleic acid sequence
caggtgcagctgcaggagtctggaggaggattggtgcaggctggggggtctctgagactctcctgcgcagtttctggaaccaccagcagtttcaatgtcatgaactggcaccaccaggctccagggaagcagcgcgagtcggtcgcaagtattactagtggtggtagcacactttatagagactccgtgaagggccgcctcaccatctccagagacaacgccaagaacgcggtgtatctgcaaatgaacagcctgaaacctgaggacacaggcgtctattactgtgggggagtagtcggtgggcgagtctactggggccaggggacccaggtcaccgtctccagcggccgctacccgtacgacgttccggactacggttccggccgagcatag

SEQ ID NO: 103 - DNA, 393 bp, Artificial Sequence
  R2DP62 nucleic acid sequence
caggtgcagctgcaggagtctgggggaggcttggtgcaggctggggggtctctgagactctcctgtgcagcctcgggaagcatcgtcagtagcaatgccatgagctggtaccgccaggctccagggaagcagcgcgagtcggtcgcagctattgcgaatagtggcataacaacgtatcgagactccgtgaagggccgattcaccatctccagagacaacaccaagaacacaatgtatctgcaaatgaacagtctgagacctgaagacacggccgtctattactgtgcagccatttttaatcaacaatttgcttggggccaggggacccaggtcaccgtctccagcggccgctacccgtacgacgttccggactacggttccggccgagcatag

SEQ ID NO: 104 - DNA, 381 bp, Artificial Sequence
  R2DP35 nucleic acid sequence
caggtgcagctgcaggagtctgggggaggcttggtgcagcctggggggtctctgacactctcctgtgccgcctctggagtcatgttcagtaccggtgtcatgggctggtaccgtcaggctccagggaagcagcgcgaggcggttgcagccattactagcggcggtctcacaacctataaagactccgtgaagggccgattcgccatctccagagacaacaccaagagtacggggtatctgcaaatgaaccgcctgagacctgaggacacggccgtctattactgcaatgtccggggctactggggtcaggggacccaggtcaccgtctccagcggccgctacccgtacgacgttccggactacggttccggccgagcatag

SEQ ID NO: 105 - DNA, 420 bp, Artificial Sequence
  R2DP55 nucleic acid sequence
caggtgcagctgcaggagtctgggggaggcttggtgcaggctggggggtctctgagagtctcctgtgcaacctctggattcactttcgatgaccatgcaataggctggttccgccaggccccagggaaggagcgcgaggcggtctcatgtcttagtaatagtgatggtactacatactatacagactccgtgaagggccgattcaccgcctccagtgacaacgccaagaaaacggggtatctacaaatgaagagcctgaaacctgaggacacggccgtttattactgtgcaatttgccattttagggaaagggacggcagtgcctggtttgagggttcctggggccaggggacccaggtcaccgtctccagcggccgctacccgtacgacgttccggactacggttccggccgagcatag

SEQ ID NO: 106 - DNA, 22 bp, Artificial Sequence
  Primer for CALL001
gtcctggctctcttctacaagg

SEQ ID NO: 107 - DNA, 23 bp, Artificial Sequence
  primer for CALL002
ggtacgtgctgttgaactgttcc

SEQ ID NO: 108 - DNA, 35 bp, Artificial Sequence
  VHH-For  primer  38
ggactagtgcggccgctggagacggtgacctgggt

SEQ ID NO: 109 - DNA, 29 bp, Artificial Sequence
  VHH-Back  primer A6E
gatgtgcagctgcaggagtctggrggagg